European Patent Application EP 4 276 112 A1, published November 15, 2023. Title: Anti-FGFR3 Antibody and Use Thereof. Applicant: AimedBio Inc. The sequence listing filed with the application follows.

SEQUENCE LISTING (219 sequences)

SEQ ID NO: 1 - protein, 5 aa, Artificial Sequence
  VH CDR1
SYYMS

SEQ ID NO: 2 - protein, 5 aa, Artificial Sequence
  VH CDR1
DYYMS

SEQ ID NO: 3 - protein, 5 aa, Artificial Sequence
  VH CDR1
GYAMS

SEQ ID NO: 4 - protein, 5 aa, Artificial Sequence
  VH CDR1
NYYMS

SEQ ID NO: 5 - protein, 5 aa, Artificial Sequence
  VH CDR1
SYDMS

SEQ ID NO: 6 - protein, 5 aa, Artificial Sequence
  VH CDR1
DYDMS

SEQ ID NO: 7 - protein, 5 aa, Artificial Sequence
  VH CDR1
NYAIH

SEQ ID NO: 8 - protein, 5 aa, Artificial Sequence
  VH CDR1
NYWIG

SEQ ID NO: 9 - protein, 5 aa, Artificial Sequence
  VH CDR1
DIAMH

SEQ ID NO: 10 - protein, 5 aa, Artificial Sequence
  VH CDR1
SYAIS

SEQ ID NO: 11 - protein, 5 aa, Artificial Sequence
  VH CDR1
IYGMH

SEQ ID NO: 12 - protein, 5 aa, Artificial Sequence
  VH CDR1
NYWMT

SEQ ID NO: 13 - protein, 5 aa, Artificial Sequence
  VH CDR1
NYPMS

SEQ ID NO: 14 - protein, 5 aa, Artificial Sequence
  VH CDR1
SYAMS

SEQ ID NO: 15 - protein, 5 aa, Artificial Sequence
  VH CDR1
GYDMS

SEQ ID NO: 16 - protein, 5 aa, Artificial Sequence
  VH CDR1
NYDMS

SEQ ID NO: 17 - protein, 5 aa, Artificial Sequence
  VH CDR1
GYYMS

SEQ ID NO: 18 - protein, 5 aa, Artificial Sequence
  VH CDR1
NYAMS

SEQ ID NO: 19 - protein, 17 aa, Artificial Sequence
  VH CDR2
AISPGSSNKYYADSVKG

SEQ ID NO: 20 - protein, 17 aa, Artificial Sequence
  VH CDR2
AIYHGDGSTYYADSVKG

SEQ ID NO: 21 - protein, 17 aa, Artificial Sequence
  VH CDR2
AISHGGSSKYYADSVKG

SEQ ID NO: 22 - protein, 17 aa, Artificial Sequence
  VH CDR2
GISPGSGSIYYADSVKG

SEQ ID NO: 23 - protein, 17 aa, Artificial Sequence
  VH CDR2
GIYSGDGSIYYADSVKG

SEQ ID NO: 24 - protein, 17 aa, Artificial Sequence
  VH CDR2
GIYYGSGNIYYADSVKG

SEQ ID NO: 25 - protein, 17 aa, Artificial Sequence
  VH CDR2
AISSSDGSTYYADSVKG

SEQ ID NO: 26 - protein, 17 aa, Artificial Sequence
  VH CDR2
SIIPISGTANYAQKFQG

SEQ ID NO: 27 - protein, 17 aa, Artificial Sequence
  VH CDR2
IIHPGGSDSRYSPSFQG

SEQ ID NO: 28 - protein, 16 aa, Artificial Sequence
  VH CDR2
TIYSSDSTYYNPSLKG

SEQ ID NO: 29 - protein, 16 aa, Artificial Sequence
  VH CDR2
SIYYSGSTYYNPSLKS

SEQ ID NO: 30 - protein, 16 aa, Artificial Sequence
  VH CDR2
SIYYTGDTYSNPSLKS

SEQ ID NO: 31 - protein, 16 aa, Artificial Sequence
  VH CDR2
SIYYSGDTYYNPSLES

SEQ ID NO: 32 - protein, 17 aa, Artificial Sequence
  VH CDR2
WINTYSGNTNYNPSLKT

SEQ ID NO: 33 - protein, 17 aa, Artificial Sequence
  VH CDR2
GINWRGATTAYADSLKG

SEQ ID NO: 34 - protein, 17 aa, Artificial Sequence
  VH CDR2
SVSGSGTSTYYADSVKG

SEQ ID NO: 35 - protein, 17 aa, Artificial Sequence
  VH CDR2
GVSYSGNNKYYADSLQS

SEQ ID NO: 36 - protein, 17 aa, Artificial Sequence
  VH CDR2
GIYPDDGSIYYADSVKG

SEQ ID NO: 37 - protein, 17 aa, Artificial Sequence
  VH CDR2
VISPSGGNIYYADSVKG

SEQ ID NO: 38 - protein, 17 aa, Artificial Sequence
  VH CDR2
VIFHDSGNIYYADSVKG

SEQ ID NO: 39 - protein, 17 aa, Artificial Sequence
  VH CDR2
AISSGGGNTYYADSVKG

SEQ ID NO: 40 - protein, 17 aa, Artificial Sequence
  VH CDR2
GISSDNSSKYYADSVKG

SEQ ID NO: 41 - protein, 17 aa, Artificial Sequence
  VH CDR2
VIYHNGSSKYYADSVKG

SEQ ID NO: 42 - protein, 7 aa, Artificial Sequence
  VH CDR3
DWSKFDY

SEQ ID NO: 43 - protein, 18 aa, Artificial Sequence
  VH CDR3
DSRLCQTSGCYSDDAMDV

SEQ ID NO: 44 - protein, 18 aa, Artificial Sequence
  VH CDR3
SRLESPFLAQSYAYAMDV

SEQ ID NO: 45 - protein, 7 aa, Artificial Sequence
  VH CDR3
DWTRFDY

SEQ ID NO: 46 - protein, 12 aa, Artificial Sequence
  VH CDR3
DAPTNEMSRFDY

SEQ ID NO: 47 - protein, 7 aa, Artificial Sequence
  VH CDR3
GGGGFDY

SEQ ID NO: 48 - protein, 7 aa, Artificial Sequence
  VH CDR3
HLPNFDY

SEQ ID NO: 49 - protein, 7 aa, Artificial Sequence
  VH CDR3
GGYGFDY

SEQ ID NO: 50 - protein, 7 aa, Artificial Sequence
  VH CDR3
WRAWFDS

SEQ ID NO: 51 - protein, 12 aa, Artificial Sequence
  VH CDR3
GVGYTTSSRFDY

SEQ ID NO: 52 - protein, 7 aa, Artificial Sequence
  VH CDR3
GASWMDM

SEQ ID NO: 53 - protein, 8 aa, Artificial Sequence
  VH CDR3
GYATALDY

SEQ ID NO: 54 - protein, 10 aa, Artificial Sequence
  VH CDR3
DIGSSWGFDY

SEQ ID NO: 55 - protein, 7 aa, Artificial Sequence
  VH CDR3
GRGMFDY

SEQ ID NO: 56 - protein, 8 aa, Artificial Sequence
  VH CDR3
SDYGLFDI

SEQ ID NO: 57 - protein, 10 aa, Artificial Sequence
  VH CDR3
HTQRWGAFDP

SEQ ID NO: 58 - protein, 8 aa, Artificial Sequence
  VH CDR3
NRNAIFDY

SEQ ID NO: 59 - protein, 18 aa, Artificial Sequence
  VH CDR3
DPLIYELPIGYSSYGMDV

SEQ ID NO: 60 - protein, 12 aa, Artificial Sequence
  VH CDR3
GPNSHIYPYFYY

SEQ ID NO: 61 - protein, 18 aa, Artificial Sequence
  VH CDR3
GILFMTITLPYSSDGMDV

SEQ ID NO: 62 - protein, 18 aa, Artificial Sequence
  VH CDR3
HPLLSIFSLPYYSDAMDV

SEQ ID NO: 63 - protein, 7 aa, Artificial Sequence
  VH CDR3
KWPTFDY

SEQ ID NO: 64 - protein, 7 aa, Artificial Sequence
  VH CDR3
DWEQFDY

SEQ ID NO: 65 - protein, 18 aa, Artificial Sequence
  VH CDR3
HTVIEALEAAYYDDGMDV

SEQ ID NO: 66 - protein, 18 aa, Artificial Sequence
  VH CDR3
HGGDETNYFQSYYDGMDV

SEQ ID NO: 67 - protein, 13 aa, Artificial Sequence
  VL CDR1
SGSSSNIGSNDVT

SEQ ID NO: 68 - protein, 13 aa, Artificial Sequence
  VL CDR1
TGSSSNIGNNYVS

SEQ ID NO: 69 - protein, 13 aa, Artificial Sequence
  VL CDR1
SGSSSNIGNNDVS

SEQ ID NO: 70 - protein, 13 aa, Artificial Sequence
  VL CDR1
TGSSSNIGNNAVS

SEQ ID NO: 71 - protein, 13 aa, Artificial Sequence
  VL CDR1
SGSSSNIGNNYVS

SEQ ID NO: 72 - protein, 13 aa, Artificial Sequence
  VL CDR1
SGSSSNIGNNDVY

SEQ ID NO: 73 - protein, 13 aa, Artificial Sequence
  VL CDR1
TGSSSNIGNNTVS

SEQ ID NO: 74 - protein, 11 aa, Artificial Sequence
  VL CDR1
RASQSISTFLN

SEQ ID NO: 75 - protein, 11 aa, Artificial Sequence
  VL CDR1
RASQSITDYLA

SEQ ID NO: 76 - protein, 11 aa, Artificial Sequence
  VL CDR1
RASQSISSYLN

SEQ ID NO: 77 - protein, 11 aa, Artificial Sequence
  VL CDR1
QASQDISNYLN

SEQ ID NO: 78 - protein, 13 aa, Artificial Sequence
  VL CDR1
SGSSSNIGSNTVN

SEQ ID NO: 79 - protein, 13 aa, Artificial Sequence
  VL CDR1
TAAASDIASNYVQ

SEQ ID NO: 80 - protein, 10 aa, Artificial Sequence
  VL CDR1
SDNIGSKSVH

SEQ ID NO: 81 - protein, 11 aa, Artificial Sequence
  VL CDR1
GGNNIGSKSVH

SEQ ID NO: 82 - protein, 11 aa, Artificial Sequence
  VL CDR1
GGDNIGTKSVH

SEQ ID NO: 83 - protein, 11 aa, Artificial Sequence
  VL CDR1
SRNNIGSKSMH

SEQ ID NO: 84 - protein, 13 aa, Artificial Sequence
  VL CDR1
SGSSSNIGSNDVN

SEQ ID NO: 85 - protein, 13 aa, Artificial Sequence
  VL CDR1
SGSSSNIGSNAVT

SEQ ID NO: 86 - protein, 13 aa, Artificial Sequence
  VL CDR1
TGSSSNIGNNDVS

SEQ ID NO: 87 - protein, 13 aa, Artificial Sequence
  VL CDR1
TGSSSNIGSNTVY

SEQ ID NO: 88 - protein, 13 aa, Artificial Sequence
  VL CDR1
SGSSSNIGSNTFN

SEQ ID NO: 89 - protein, 7 aa, Artificial Sequence
  VL CDR2
DDNHRPS

SEQ ID NO: 90 - protein, 7 aa, Artificial Sequence
  VL CDR2
YNSHRPS

SEQ ID NO: 91 - protein, 7 aa, Artificial Sequence
  VL CDR2
SNSHRPS

SEQ ID NO: 92 - protein, 7 aa, Artificial Sequence
  VL CDR2
DDSKRPS

SEQ ID NO: 93 - protein, 7 aa, Artificial Sequence
  VL CDR2
ADSKRPS

SEQ ID NO: 94 - protein, 7 aa, Artificial Sequence
  VL CDR2
ADNHRPS

SEQ ID NO: 95 - protein, 7 aa, Artificial Sequence
  VL CDR2
YDSHRPS

SEQ ID NO: 96 - protein, 7 aa, Artificial Sequence
  VL CDR2
DATNRAT

SEQ ID NO: 97 - protein, 7 aa, Artificial Sequence
  VL CDR2
DASNRAT

SEQ ID NO: 98 - protein, 7 aa, Artificial Sequence
  VL CDR2
DASNRAA

SEQ ID NO: 99 - protein, 7 aa, Artificial Sequence
  VL CDR2
DTSNKHS

SEQ ID NO: 100 - protein, 7 aa, Artificial Sequence
  VL CDR2
EDTKRPS

SEQ ID NO: 101 - protein, 7 aa, Artificial Sequence
  VL CDR2
SNNQRPS

SEQ ID NO: 102 - protein, 7 aa, Artificial Sequence
  VL CDR2
QDTKRPS

SEQ ID NO: 103 - protein, 7 aa, Artificial Sequence
  VL CDR2
GNSNRPS

SEQ ID NO: 104 - protein, 7 aa, Artificial Sequence
  VL CDR2
DNNKRPS

SEQ ID NO: 105 - protein, 7 aa, Artificial Sequence
  VL CDR2
YDSNRPS

SEQ ID NO: 106 - protein, 7 aa, Artificial Sequence
  VL CDR2
SDNHRPS

SEQ ID NO: 107 - protein, 7 aa, Artificial Sequence
  VL CDR2
ANNQRPS

SEQ ID NO: 108 - protein, 7 aa, Artificial Sequence
  VL CDR2
SNSQRPS

SEQ ID NO: 109 - protein, 7 aa, Artificial Sequence
  VL CDR2
SDSNRPS

SEQ ID NO: 110 - protein, 11 aa, Artificial Sequence
  VL CDR3
GTWDASLSAYV

SEQ ID NO: 111 - protein, 11 aa, Artificial Sequence
  VL CDR3
ATWDDSLSGYV

SEQ ID NO: 112 - protein, 11 aa, Artificial Sequence
  VL CDR3
GTWDDSLNGYV

SEQ ID NO: 113 - protein, 11 aa, Artificial Sequence
  VL CDR3
GAWDYSLSAYV

SEQ ID NO: 114 - protein, 11 aa, Artificial Sequence
  VL CDR3
ASWDYSLSGYV

SEQ ID NO: 115 - protein, 11 aa, Artificial Sequence
  VL CDR3
GAWDASLNGYV

SEQ ID NO: 116 - protein, 9 aa, Artificial Sequence
  VL CDR3
QQANSFPLT

SEQ ID NO: 117 - protein, 9 aa, Artificial Sequence
  VL CDR3
QQSYSTPFT

SEQ ID NO: 118 - protein, 10 aa, Artificial Sequence
  VL CDR3
CQQYSSFPLT

SEQ ID NO: 119 - protein, 9 aa, Artificial Sequence
  VL CDR3
QQSYSTPIT

SEQ ID NO: 120 - protein, 11 aa, Artificial Sequence
  VL CDR3
AAWDNSLNGQL

SEQ ID NO: 121 - protein, 11 aa, Artificial Sequence
  VL CDR3
ATWDDSLRGWV

SEQ ID NO: 122 - protein, 9 aa, Artificial Sequence
  VL CDR3
QSYDSSTVV

SEQ ID NO: 123 - protein, 9 aa, Artificial Sequence
  VL CDR3
QSYDSRQLV

SEQ ID NO: 124 - protein, 11 aa, Artificial Sequence
  VL CDR3
QSYDSSLSGYV

SEQ ID NO: 125 - protein, 10 aa, Artificial Sequence
  VL CDR3
SSYTSSSTLV

SEQ ID NO: 126 - protein, 11 aa, Artificial Sequence
  VL CDR3
AAWDSSLSGYV

SEQ ID NO: 127 - protein, 11 aa, Artificial Sequence
  VL CDR3
GTWDYSLSGYV

SEQ ID NO: 128 - protein, 11 aa, Artificial Sequence
  VL CDR3
GAWDDSLSAYV

SEQ ID NO: 129 - protein, 11 aa, Artificial Sequence
  VL CDR3
GAWDSSLNAYV

SEQ ID NO: 130 - protein, 11 aa, Artificial Sequence
  VL CDR3
GTWDDSLSGYV

SEQ ID NO: 131 - protein, 11 aa, Artificial Sequence
  VL CDR3
GAWDSSLSAYV

SEQ ID NO: 132 - protein, 11 aa, Artificial Sequence
  VL CDR3
GTWDYSLNGYV

SEQ ID NO: 133 - protein, 116 aa, Artificial Sequence
  VH
EVQLLESGGGLVQPGGSLRLSCAASGFTFSSYYMSWVRQAPGKGLEWVSAISPGSSNKYYADSVKGRFTISRDNSKNTLYLQMNSLRAEDTAVYYCAKDWSKFDYWGQGTLVTVSS

SEQ ID NO: 134 - protein, 127 aa, Artificial Sequence
  VH
EVQLLESGGGLVQPGGSLRLSCAASGFTFSDYYMSWVRLAPGKGLEWVSAIYHGDGSTYYADSVKGRFTISRDNSKNTLYLQMNSLRAEDTAVYYCARDSRLCQTSGCYSDDAMDVWGQGTLVTVSS

SEQ ID NO: 135 - protein, 127 aa, Artificial Sequence
  VH
EVQLLESGGGLVQPGGSLRLSCAASGFTFSGYAMSWVRQAPGKGLEWVSAISHGGSSKYYADSVKGRFTISRDNSKNTLYLQMNSLRAEDTAVYYCARSRLESPFLAQSYAYAMDVWGQGTLVTVSS

SEQ ID NO: 136 - protein, 116 aa, Artificial Sequence
  VH
EVQLLESGGGLVQPGGSLRLSCAASGFTFSNYYMSWVRQAPGKGLEWVSGISPGSGSIYYADSVKGRFTISRDNSKNTLYLQMNSLRAEDTAVYYCAKDWTRFDYWGQGTLVTVSS

SEQ ID NO: 137 - protein, 121 aa, Artificial Sequence
  VH
EVQLLESGGGLVQPGGSLRLSCAASGFTFSSYDMSWVRQAPGKGLEWVSGIYSGDGSIYYADSVKGRFTISRDNSKNTLYLQMNSLRAEDTAVYYCAKDAPTNEMSRFDYWGQGTLVTVSS

SEQ ID NO: 138 - protein, 116 aa, Artificial Sequence
  VH
EVQLLESGGGLVQPGGSLRLSCAASGFTFSNYYMSWVRQAPGKGLEWVSGIYYGSGNIYYADSVKGRFTISRDNSKNTLYLQMNSLRAEDTAVYYCARGGGGFDYWGQGTLVTVSS

SEQ ID NO: 139 - protein, 116 aa, Artificial Sequence
  VH
EVQLLESGGGLVQPGGSLRLSCAASGFTFSDYDMSWVRQAPGKGLEWVSAISSSDGSTYYADSVKGRFTISRDNSKNTLYLQMNSLRAEDTAVYYCAKHLPNFDYWGQGTLVTVSS

SEQ ID NO: 140 - protein, 116 aa, Artificial Sequence
  VH
EVQLLESGGGLVQPGGSLRLSCAASGFTFSNYAIHWVRQAPGKGLEWVSSIIPISGTANYAQKFQGRFTISRDNSKNTLYLQMNSLRAEDTAVYYCSRGGYGFDYWGQGTLVTVSS

SEQ ID NO: 141 - protein, 116 aa, Artificial Sequence
  VH
EVQLLESGGGLVQPGGSLRLSCAASGFTFSNYWIGWVRQAPGKGLEWVSIIHPGGSDSRYSPSFQGRFTISRDNSKNTLYLQMNSLRAEDTAVYYCARWRAWFDSWGQGTLVTVSS

SEQ ID NO: 142 - protein, 120 aa, Artificial Sequence
  VH
EVQLLESGGGLVQPGGSLRLSCAASRFTFSDIAMHWVRQAPGKGLEWVSTIYSSDSTYYNPSLKGRFTISRDNSKNTLYLQMNSLRAEDTAVYYCAKGVGYTTSSRFDYWGQGTLVTVSS

SEQ ID NO: 143 - protein, 115 aa, Artificial Sequence
  VH
EVQLLESGGGLVQPGGSLRLSCAASGFTFSSYAISWVRQAPGKGLEWVSSIYYSGSTYYNPSLKSRFTISRDNSKNTLYLQMNSLRAEDTAVYYCAQGASWMDMWGQGTLVTVSS

SEQ ID NO: 144 - protein, 116 aa, Artificial Sequence
  VH
EVQLLESGGGLVQPGGSLRLSCAASGFTFSIYGMHWVRQAPGKGLEWVSSIYYTGDTYSNPSLKSRFTISRDNSKNTLYLQMNSLRAEDTAVYYCARGYATALDYWGQGTLVTVSS

SEQ ID NO: 145 - protein, 118 aa, Artificial Sequence
  VH
EVQLLESGGGLVQPGGSLRLSCAASGFTFSIYGMHWVRQAPGKGLEWVSSIYYSGDTYYNPSLESRFTISRDNSKNTLYLQMNSLRAEDTAVYYCARDIGSSWGFDYWGQGTLVTVSS

SEQ ID NO: 146 - protein, 116 aa, Artificial Sequence
  VH
EVQLLESGGGLVQPGGSLRLSCAASGFTFSNYWMTWVRQAPGKGLEWVSWINTYSGNTNYNPSLKTRFTISRDNSKNTLYLQMNSLRAEDTAVYYCARGRGMFDYWGQGTLVTVSS

SEQ ID NO: 147 - protein, 117 aa, Artificial Sequence
  VH
EVQLLESGGGLVQPGGSLRLSCAASGFTFSGYAMSWVRQAPGKGLEWVSGINWRGATTAYADSLKGRFTISRDNSKNTLYLQMNSLRAEDTAVYYCARSDYGLFDIWGQGTLVTVSS

SEQ ID NO: 148 - protein, 119 aa, Artificial Sequence
  VH
EVQLLESGGGLVQPGGSLRLSCAASGFTFSNYPMSWVRQAPGKGLEWVSSVSGSGTSTYYADSVKGRFTISRDNSKNTLHLQMNSLRAEDTAVYYCARHTQRWGAFDPWGQGTLVTVSS

SEQ ID NO: 149 - protein, 117 aa, Artificial Sequence
  VH
EVQLLESGGGLVQPGGSLRLSCAASGFTFSSYAMSWVRQAPGKGLEWVSGVSYSGNNKYYADSLQSRFTISRDNSKNTLYLQMNSLRAEDTAVYYCARNRNAIFDYWGQGTLVTVSS

SEQ ID NO: 150 - protein, 127 aa, Artificial Sequence
  VH
EVQLLESGGGLVQPGGSLRLSCAASGFTFSSYYMSWVRQAPGKGLEWVSGIYPDDGSIYYADSVKGRFTISRDNSKNTLYLQMNSLRAEDTAVYYCAKDPLIYELPIGYSSYGMDVWGQGTLVTVSS

SEQ ID NO: 151 - protein, 121 aa, Artificial Sequence
  VH
EVQLLESGGGLVQPGGSLRLSCAASGFTFSDYDMSWVRQAPGKGLEWVSGIYSGDGSIYYADSVKGRFTISRDNSKNTLYLQMNSLRAEDTAVYYCAKGPNSHIYPYFYYWGQGTLVTVSS

SEQ ID NO: 152 - protein, 127 aa, Artificial Sequence
  VH
EVQLLESGGGLVQPGGSLRLSCAASGFTFSGYDMSWVRQAPGKGLEWVSVISPSGGNIYYADSVKGRFTISRDNSKNTLYLQMNSLRAEDTAVYYCARGILFMTITLPYSSDGMDVWGQGTLVTVSS

SEQ ID NO: 153 - protein, 127 aa, Artificial Sequence
  VH
EVQLLESGGGLVQPGGSLRLSCAASGFTFSNYDMSWVRQAPGKGLEWVSVIFHDSGNIYYADSVKGRFTISRDNSKNTLYLQMNSLRAEDTAVYYCAKHPLLSIFSLPYYSDAMDVWGQGTLVTVSS

SEQ ID NO: 154 - protein, 116 aa, Artificial Sequence
  VH
EVQLLESGGGLVQPGGSLRLSCAASGFTFSGYYMSWVRQAPGKGLEWVSAISSGGGNTYYADSVKGRFTISRDNSKNTLYLQMNSLRAEDTAVYYCARKWPTFDYWGQGTLVTVSS

SEQ ID NO: 155 - protein, 116 aa, Artificial Sequence
  VH
EVQLLESGGGLVQPGGSLRLSCAASGFTFSNYYMSWVRQAPGKGLEWVSAISPGSSNKYYADSVKGRFTISRDNSKNTLYLQMNSLRAEDTAVYYCAKDWEQFDYWGQGTLVTVSS

SEQ ID NO: 156 - protein, 127 aa, Artificial Sequence
  VH
EVQLLESGGGLVQPGGSLRLSCAASGFTFSNYAMSWVRQAPGKGLEWVSGISSDNSSKYYADSVKGRFTISRDNSKNTLYLQMNSLRAEDTAVYYCAKHTVIEALEAAYYDDGMDVWGQGTLVTVSS

SEQ ID NO: 157 - protein, 127 aa, Artificial Sequence
  VH
EVQLLESGGGLVQPGGSLRLSCAASGFTFSNYDMSWVRQAPGKGLEWVSVIYHNGSSKYYADSVKGRFTISRDNSKNTLYLQMNSLRAEDTAVYYCAKHGGDETNYFQSYYDGMDVWGQGTLVTVSS

SEQ ID NO: 158 - protein, 110 aa, Artificial Sequence
  VL
QSVLTQPPSASGTPGQRVTISCSGSSSNIGSNDVTWYQQLPGTAPKLLIYDDNHRPSGVPDRFSGSKSGTSASLAISGLRSEDEADYYCGTWDASLSAYVFGGGTKLTVL

SEQ ID NO: 159 - protein, 110 aa, Artificial Sequence
  VL
QSVLTQPPSASGTPGQRVTISCTGSSSNIGNNYVSWYQQLPGTAPKLLIYYNSHRPSGVPDRFSGSKSGTSASLAISGLRSEDEADYYCATWDDSLSGYVFGGGTKLTVL

SEQ ID NO: 160 - protein, 110 aa, Artificial Sequence; identical to SEQ ID NO: 159
  VL

SEQ ID NO: 161 - protein, 110 aa, Artificial Sequence
  VL
QSVLTQPPSASGTPGQRVTISCTGSSSNIGNNAVSWYQQLPGTAPKLLIYDDSKRPSGVPDRFSGSKSGTSASLAISGLRSEDEADYYCGAWDYSLSAYVFGGGTKLTVL

SEQ ID NO: 162 - protein, 110 aa, Artificial Sequence
  VL
QSVLTQPPSASGTPGQRVTISCSGSSSNIGNNYVSWYQQLPGTAPKLLIYADSKRPSGVPDRFSGSKSGTSASLAISGLRSEDEADYYCASWDYSLSGYVFGGGTKLTVL

SEQ ID NO: 163 - protein, 110 aa, Artificial Sequence
  VL
QSVLTQPPSASGTPGQRVTISCSGSSSNIGNNDVYWYQQLPGTAPKLLIYADNHRPSGVPDRFSGSKSGTSASLAISGLRSEDEADYYCGAWDASLNGYVFGGGTKLTVL

SEQ ID NO: 164 - protein, 110 aa, Artificial Sequence
  VL
QSVLTQLPSASGTPGQRVTISCTGSSSNIGNNTVSWYQQLPGTAPKLLIYYDSHRPSGVPDRFSGSKSGTSASLAISGLRSEDEADYYCGTWDDSLNGYVFGGGTKLTVL

SEQ ID NO: 165 - protein, 107 aa, Artificial Sequence
  VL
EIVLTQSPGTLSLSPGERATLSCRASQSISTFLNWYQQKPGQAPRLLIYDATNRATGIPDRFSGSGSGTDFTLTISRLEPEDFAVYYCQQANSFPLTFGQGTKVEIK

SEQ ID NO: 166 - protein, 107 aa, Artificial Sequence
  VL
EIVLTQSPGTLSLSPGERATLSCRASQSITDYLAWYQQKPGQAPRLLIYDASNRATGIPDRFSGSGSGTDFTLTISRLEPEDFAVYYCQQSYSTPFTFGQGTKVEIK

SEQ ID NO: 167 - protein, 107 aa, Artificial Sequence
  VL
EIVLTQGPGTLSLSPGERATLSCRASQSISSYLNWYQQKPGQAPRLLVYDASNRAAGIPDRFSGSGSGTDFTLTISRLEPEDFAVYYCQQYSSFPLTFGQGTKVEIK

SEQ ID NO: 168 - protein, 107 aa, Artificial Sequence
  VL
EIVLTQSPGTLSLSPGERATLSCQASQDISNYLNWYQQKPGQAPRLLIYDASNRATGIPDRFSGSGSGTDFTLTISRLEPEDFAVYYCQQSYSTPITFGQGTKVEIK

SEQ ID NO: 169 - protein, 108 aa, Artificial Sequence
  VL
QSVLTQPPSASGTPGQRVTISCSGSSSNIGSNTVNWYQQLPGTAPKLLIYDTSNKHSGDRFSGSKSGTSASLAISGLRSEDEADYYCAAWDNSLNGQLFGGGTKLTVL

SEQ ID NO: 170 - protein, 110 aa, Artificial Sequence
  VL
QSVLTQPPSASGTPGQRVTISCTAAASDIASNYVQWYQQLPGTAPKLLIYEDTKRPSGVPYRFSGSKSGTSASLAISGLRSEDEADYYCATWDDSLRGWVFGGGTKLTVL

SEQ ID NO: 171 - protein, 105 aa, Artificial Sequence
  VL
QSVLTQPPSASGTPGQRVTISCSDNIGSKSVHWYQQLPGTAPKLLIYSNNQRPSGVSDRFSGSKSGTSASLAISGLRSEDEADYYCQSYDSSTVVFGGGTKLTVL

SEQ ID NO: 172 - protein, 106 aa, Artificial Sequence
  VL
QSVLTQPPSASGAPGQRVTISCGGNNIGSKSVHWYQQLPGTAPKLLIYQDTKRPSGVPNRFSGSKSGTSASLAISGLRSEDEADYYCQSYDSRQLVFGGGTKLTVL

SEQ ID NO: 173 - protein, 108 aa, Artificial Sequence
  VL
QSVLTQPPSASGTPGQRVTISCGGDNIGTKSVHWYQQLPGTAPKLLIYGNSNRPSGVPNRFSGSKSGTSASLAISGLRSEDEADYYCQSYDSSLSGYVFGGGTKLTVL

SEQ ID NO: 174 - protein, 107 aa, Artificial Sequence
  VL
QSVLTQPPSASATPGQRVTISCSRNNIGSKSMHWYQQLPGTAPKLLIYDNNKRPSGVSDRFSGSKSGTSASLAISGLRSEDEADYYCSSYTSSSTLVFGGGTKLTVL

SEQ ID NO: 175 - protein, 110 aa, Artificial Sequence
  VL
QSVLTQPPSASGTPGQRVTISCSGSSSNIGSNDVNWYQQLPGTAPKLLIYYDSNRPSGVPDRFSGSKSGTSASLAISGLRSEDEADYYCAAWDSSLSGYVFGGGTKLTVL

SEQ ID NO: 176 - protein, 110 aa, Artificial Sequence
  VL
QSVLTQPPSASGTPGQRVTISCSGSSSNIGNNDVSWYQQLPGTAPKLLIYSNSHRPSGVPDRFSGSKSGTSASLAISGLRSEDEADYYCGTWDYSLSGYVFGGGTKLTVL

SEQ ID NO: 177 - protein, 110 aa, Artificial Sequence
  VL
QSVLTQPPSASGTPGQRVTISCSGSSSNIGSNAVTWYQQLPGTAPKLLIYDDNHRPSGVPDRFSGSKSGTSASLAISGLRSEDEADYYCGAWDDSLSAYVFGGGTKLTVL

SEQ ID NO: 178 - protein, 110 aa, Artificial Sequence
  VL
QSVLTQPPSASGTPGQRVTISCTGSSSNIGNNDVSWYQQLPGTAPKLLIYSDNHRPSGVPDRFSGSKSGTSASLAISGLRSEDEADYYCGAWDSSLNAYVFGGGTKLTVL

SEQ ID NO: 179 - protein, 110 aa, Artificial Sequence
  VL
QSVLTQPPSASGTPGQRVTISCTGSSSNIGSNTVYWYQQLPGTAPKLLIYANNQRPSGVPDRFSGSKSGTSASLAISGLRSEDEADYYCGTWDDSLSGYVFGGGTKLTVL

SEQ ID NO: 180 - protein, 110 aa, Artificial Sequence
  VL
QSVLTQPPSASGTPGQRVTISCSGSSSNIGSNTFNWYQQLPGTAPKLLIYSNSQRPSGVPDRFSGSKSGTSASLAISGLRSEDEADYYCGAWDSSLSAYVFGGGTKLTVL

SEQ ID NO: 181 - protein, 110 aa, Artificial Sequence; identical to SEQ ID NO: 177
  VL

SEQ ID NO: 182 - protein, 110 aa, Artificial Sequence
  VL
QSVLTQPPSASGTPGQRVTISCSGSSSNIGNNDVYWYQQLPGTAPKLLIYSDSNRPSGVPDRFSGSKSGTSASLAISGLRSEDEADYYCGTWDYSLNGYVFGGGTKLTVL

SEQ ID NO: 183 - protein, 806 aa, Artificial Sequence
  FGFR3
MGAPACALALCVAVAIVAGASSESLGTEQRVVGRAAEVPGPEPGQQEQLVFGSGDAVELSCPPPGGGPMGPTVWVKDGTGLVPSERVLVGPQRLQVLNASHEDSGAYSCRQRLTQRVLCHFSVRVTDAPSSGDDEDGEDEAEDTGVDTGAPYWTRPERMDKKLLAVPAANTVRFRCPAAGNPTPSISWLKNGREFRGEHRIGGIKLRHQQWSLVMESVVPSDRGNYTCVVENKFGSIRQTYTLDVLERSPHRPILQAGLPANQTAVLGSDVEFHCKVYSDAQPHIQWLKHVEVNGSKVGPDGTPYVTVLKTAGANTTDKELEVLSLHNVTFEDAGEYTCLAGNSIGFSHHSAWLVVLPAEEELVEADEAGSVYAGILSYGVGFFLFILVVAAVTLCRLRSPPKKGLGSPTVHKISRFPLKRQVSLESNASMSSNTPLVRIARLSSGEGPTLANVSELELPADPKWELSRARLTLGKPLGEGCFGQVVMAEAIGIDKDRAAKPVTVAVKMLKDDATDKDLSDLVSEMEMMKMIGKHKNIINLLGACTQGGPLYVLVEYAAKGNLREFLRARRPPGLDYSFDTCKPPEEQLTFKDLVSCAYQVARGMEYLASQKCIHRDLAARNVLVTEDNVMKIADFGLARDVHNLDYYKKTTNGRLPVKWMAPEALFDRVYTHQSDVWSFGVLLWEIFTLGGSPYPGIPVEELFKLLKEGHRMDKPANCTHDLYMIMRECWHAAPSQRPTFKQLVEDLDRVLTVTSTDEYLDLSAPFEQYSPGGQDTPSSSSSGDDSVFAHDLLPPAPPSSGGSRT

SEQ ID NO: 184 - protein, 138 aa, Artificial Sequence
  FGFR3 D1
MGAPACALALCVAVAIVAGASSESLGTEQRVVGRAAEVPGPEPGQQEQLVFGSGDAVELSCPPPGGGPMGPTVWVKDGTGLVPSERVLVGPQRLQVLNASHEDSGAYSCRQRLTQRVLCHFSVRVTDAPSSGDDEDGE

SEQ ID NO: 185 - protein, 15 aa, Artificial Sequence
  linker
GGGGSGGGGSGGGGS

SEQ ID NO: 186 - protein, 12 aa, Artificial Sequence
  VH CDR3
DYPTNEMSRFDY

SEQ ID NO: 187 - protein, 12 aa, Artificial Sequence
  VH CDR3
DGPTNEMSRFDY

SEQ ID NO: 188 - protein, 12 aa, Artificial Sequence
  VH CDR3
DAPMNEMSRFDY

SEQ ID NO: 189 - protein, 12 aa, Artificial Sequence
  VH CDR3
DAPTNEISRFDY

SEQ ID NO: 190 - protein, 12 aa, Artificial Sequence
  VH CDR3
DAPTNEPSRFDY

SEQ ID NO: 191 - protein, 12 aa, Artificial Sequence
  VH CDR3
DAPTNEESRFDY

SEQ ID NO: 192 - protein, 12 aa, Artificial Sequence
  VH CDR3
DGPMNEMSRFDY

SEQ ID NO: 193 - protein, 12 aa, Artificial Sequence
  VH CDR3
DGPTNEISRFDY

SEQ ID NO: 194 - protein, 12 aa, Artificial Sequence
  VH CDR3
DGPTNEESRFDY

SEQ ID NO: 195 - protein, 12 aa, Artificial Sequence
  VH CDR3
DAPMNEISRFDY

SEQ ID NO: 196 - protein, 12 aa, Artificial Sequence
  VH CDR3
DAPMNEESRFDY

SEQ ID NO: 197 - protein, 12 aa, Artificial Sequence
  VH CDR3
DGPMNEISRFDY

SEQ ID NO: 198 - protein, 12 aa, Artificial Sequence
  VH CDR3
DGPMNEESRFDY

SEQ ID NO: 199 - protein, 11 aa, Artificial Sequence
  VL CDR3
AVWDYSLSGYV

SEQ ID NO: 200 - protein, 11 aa, Artificial Sequence
  VL CDR3
ASWDYSLTGYV

SEQ ID NO: 201 - protein, 11 aa, Artificial Sequence
  VL CDR3
ASWDYSLDGYV

SEQ ID NO: 202 - protein, 11 aa, Artificial Sequence
  VL CDR3
ASWDYSLEGYV

SEQ ID NO: 203 - protein, 121 aa, Artificial Sequence
  VH
EVQLLESGGGLVQPGGSLRLSCAASGFTFSSYDMSWVRQAPGKGLEWVSGIYSGDGSIYYADSVKGRFTISRDNSKNTLYLQMNSLRAEDTAVYYCAKDYPTNEMSRFDYWGQGTLVTVSS

SEQ ID NO: 204 - protein, 121 aa, Artificial Sequence
  VH
EVQLLESGGGLVQPGGSLRLSCAASGFTFSSYDMSWVRQAPGKGLEWVSGIYSGDGSIYYADSVKGRFTISRDNSKNTLYLQMNSLRAEDTAVYYCAKDGPTNEMSRFDYWGQGTLVTVSS

SEQ ID NO: 205 - protein, 121 aa, Artificial Sequence
  VH
EVQLLESGGGLVQPGGSLRLSCAASGFTFSSYDMSWVRQAPGKGLEWVSGIYSGDGSIYYADSVKGRFTISRDNSKNTLYLQMNSLRAEDTAVYYCAKDAPMNEMSRFDYWGQGTLVTVSS

SEQ ID NO: 206 - protein, 121 aa, Artificial Sequence
  VH
EVQLLESGGGLVQPGGSLRLSCAASGFTFSSYDMSWVRQAPGKGLEWVSGIYSGDGSIYYADSVKGRFTISRDNSKNTLYLQMNSLRAEDTAVYYCAKDAPTNEISRFDYWGQGTLVTVSS

SEQ ID NO: 207 - protein, 121 aa, Artificial Sequence
  VH
EVQLLESGGGLVQPGGSLRLSCAASGFTFSSYDMSWVRQAPGKGLEWVSGIYSGDGSIYYADSVKGRFTISRDNSKNTLYLQMNSLRAEDTAVYYCAKDAPTNEPSRFDYWGQGTLVTVSS

SEQ ID NO: 208 - protein, 121 aa, Artificial Sequence
  VH
EVQLLESGGGLVQPGGSLRLSCAASGFTFSSYDMSWVRQAPGKGLEWVSGIYSGDGSIYYADSVKGRFTISRDNSKNTLYLQMNSLRAEDTAVYYCAKDAPTNEESRFDYWGQGTLVTVSS

SEQ ID NO: 209 - protein, 121 aa, Artificial Sequence
  VH
EVQLLESGGGLVQPGGSLRLSCAASGFTFSSYDMSWVRQAPGKGLEWVSGIYSGDGSIYYADSVKGRFTISRDNSKNTLYLQMNSLRAEDTAVYYCAKDGPMNEMSRFDYWGQGTLVTVSS

SEQ ID NO: 210 - protein, 121 aa, Artificial Sequence
  VH
EVQLLESGGGLVQPGGSLRLSCAASGFTFSSYDMSWVRQAPGKGLEWVSGIYSGDGSIYYADSVKGRFTISRDNSKNTLYLQMNSLRAEDTAVYYCAKDGPTNEISRFDYWGQGTLVTVSS

SEQ ID NO: 211 - protein, 121 aa, Artificial Sequence
  VH
EVQLLESGGGLVQPGGSLRLSCAASGFTFSSYDMSWVRQAPGKGLEWVSGIYSGDGSIYYADSVKGRFTISRDNSKNTLYLQMNSLRAEDTAVYYCAKDGPTNEESRFDYWGQGTLVTVSS

SEQ ID NO: 212 - protein, 121 aa, Artificial Sequence
  VH
EVQLLESGGGLVQPGGSLRLSCAASGFTFSSYDMSWVRQAPGKGLEWVSGIYSGDGSIYYADSVKGRFTISRDNSKNTLYLQMNSLRAEDTAVYYCAKDAPMNEISRFDYWGQGTLVTVSS

SEQ ID NO: 213 - protein, 121 aa, Artificial Sequence
  VH
EVQLLESGGGLVQPGGSLRLSCAASGFTFSSYDMSWVRQAPGKGLEWVSGIYSGDGSIYYADSVKGRFTISRDNSKNTLYLQMNSLRAEDTAVYYCAKDAPMNEESRFDYWGQGTLVTVSS

SEQ ID NO: 214 - protein, 121 aa, Artificial Sequence
  VH
EVQLLESGGGLVQPGGSLRLSCAASGFTFSSYDMSWVRQAPGKGLEWVSGIYSGDGSIYYADSVKGRFTISRDNSKNTLYLQMNSLRAEDTAVYYCAKDGPMNEISRFDYWGQGTLVTVSS

SEQ ID NO: 215 - protein, 121 aa, Artificial Sequence
  VH
EVQLLESGGGLVQPGGSLRLSCAASGFTFSSYDMSWVRQAPGKGLEWVSGIYSGDGSIYYADSVKGRFTISRDNSKNTLYLQMNSLRAEDTAVYYCAKDGPMNEESRFDYWGQGTLVTVSS

SEQ ID NO: 216 - protein, 110 aa, Artificial Sequence
  VL
QSVLTQPPSASGTPGQRVTISCSGSSSNIGNNYVSWYQQLPGTAPKLLIYADSKRPSGVPDRFSGSKSGTSASLAISGLRSEDEADYYCAVWDYSLSGYVFGGGTKLTVL

SEQ ID NO: 217 - protein, 110 aa, Artificial Sequence
  VL
QSVLTQPPSASGTPGQRVTISCSGSSSNIGNNYVSWYQQLPGTAPKLLIYADSKRPSGVPDRFSGSKSGTSASLAISGLRSEDEADYYCASWDYSLTGYVFGGGTKLTVL

SEQ ID NO: 218 - protein, 110 aa, Artificial Sequence
  VL
QSVLTQPPSASGTPGQRVTISCSGSSSNIGNNYVSWYQQLPGTAPKLLIYADSKRPSGVPDRFSGSKSGTSASLAISGLRSEDEADYYCASWDYSLDGYVFGGGTKLTVL

SEQ ID NO: 219 - protein, 110 aa, Artificial Sequence
  VL
QSVLTQPPSASGTPGQRVTISCSGSSSNIGNNYVSWYQQLPGTAPKLLIYADSKRPSGVPDRFSGSKSGTSASLAISGLRSEDEADYYCASWDYSLEGYVFGGGTKLTVL